European Patent Application EP 4 338 752 A2, published March 20, 2024. Title: Stable Liquid Pharmaceutical Preparation. Applicant: Celltrion Inc. Application EP. The sequence listing filed with the application follows.

SEQUENCE LISTING (10 sequences)

SEQ ID NO: 1 - protein, 6 aa, synthetic construct
  REGION 1..6: note = Antibody
QFVGSS

SEQ ID NO: 2 - skipped

SEQ ID NO: 3 - protein, 9 aa, synthetic construct
  REGION 1..9: note = Antibody
QQSHSWPFT

SEQ ID NO: 4 - protein, 8 aa, synthetic construct
  REGION 1..8: note = Antibody
GFIFSNHW

SEQ ID NO: 5 - protein, 10 aa, synthetic construct
  REGION 1..10: note = Antibody
IRSKSINSAT

SEQ ID NO: 6 - protein, 11 aa, synthetic construct
  REGION 1..11: note = Antibody
SRNYYGSTYDY

SEQ ID NO: 7 - protein, 107 aa, synthetic construct
  REGION 1..107: note = Antibody
DILLTQSPAILSVSPGERVSFSCRASQFVGSSIHWYQQRTNGSPRLLIKYASESMSGIPSRFSGSGSGTDFTLSINTVESEDIADYYCQQSHSWPFTFGSGTNLEVK

SEQ ID NO: 8 - protein, 119 aa, synthetic construct
  REGION 1..119: note = Antibody
EVKLEESGGGLVQPGGSMKLSCVASGFIFSNHWMNWVRQSPEKGLEWVAEIRSKSINSATHYAESVKGRFTISRDDSKSAVYLQMTDLRTEDTGVYYCSRNYYGSTYDYWGQGTTLTVS

SEQ ID NO: 9 - protein, 236 aa, synthetic construct
  REGION 1..236: note = Antibody
MDFQVQIISFLLISASVIMSRGDILLTQSPAILSVSPGERVSFSCRASQFVGSSIHWYQQRTNGSPRLLIKYASESMSGIPSRFSGSGSGTDFTLSINTVESEDIADYYCQQSHSWPFTFGSGTNLEVKRTVAAPSVFIFPPSDEQLKSGTASVVCLLNNFYPREAKVQWKVDNALQSGNSQESVTEQDSKDSTYSLSSTLTLSKADYEKHKVYACEVTHQGLSSPVTKSFNRGEC

SEQ ID NO: 10 - protein, 469 aa, synthetic construct
  REGION 1..469: note = Antibody
MGWSLILLFLVAVATRVLSEVKLEESGGGLVQPGGSMKLSCVASGFIFSNHWMNWVRQSPEKGLEWVAEIRSKSINSATHYAESVKGRFTISRDDSKSAVYLQMTDLRTEDTGVYYCSRNYYGSTYDYWGQGTTLTVSSASTKGPSVFPLAPSSKSTSGGTAALGCLVKDYFPEPVTVSWNSGALTSGVHTFPAVLQSSGLYSLSSVVTVPSSSLGTQTYICNVNHKPSNTKVDKKVEPKSCDKTHTCPPCPAPELLGGPSVFLFPPKPKDTLMISRTPEVTCVVVDVSHEDPEVKFNWYVDGVEVHNAKTKPREEQYNSTYRVVSVLTVLHQDWLNGKEYKCKVSNKALPAPIEKTISKAKGQPREPQVYTLPPSRDELTKNQVSLTCLVKGFYPSDIAVEWESNGQPENNYKTTPPVLDSDGSFFLYSKLTVDKSRWQQGNVFSCSVMHEALHNHYTQKSLSLSPGK